European Patent Application EP 4 183 801 A1, published May 24, 2023. Title: VHH antibodies against SARS-CoV-2-variants. Applicant: Max-Planck Gesellschaft zur Förderung der Wissenschaften e.V. The sequence listing filed with the application follows.

SEQUENCE LISTING (117 sequences)

SEQ ID NO: 1 - protein, 127 aa, Artificial Sequence
  Re5D06
QVQLVESGGGLVQPGGSLRLSCAASGITLDYYAIGWFRQAPGKEREGVSRIRSSDGSTNYADSVKGRFTMSRDNAKNTVYLQMNSLKPEDTAVYYCAYGPLTKYGSSWYWPYEYDYWGQGTQVTVSS

SEQ ID NO: 2 - protein, 9 aa, Artificial Sequence
  Re5D06 CDR1
ITLDYYAIG

SEQ ID NO: 3 - protein, 15 aa, Artificial Sequence
  Re5D06 CDR2
SRIRSSDGSTNYADS

SEQ ID NO: 4 - protein, 19 aa, Artificial Sequence
  Re5D06 CDR3
YGPLTKYGSSWYWPYEYDY

SEQ ID NO: 5 - protein, 127 aa, Artificial Sequence
  Re5D06R15
QVQLVESGGGLVQPGGSLRLSCAASGITLDYYAMGWFREAPGKEREGVARIRNSDGSTNYADSVKGRFTMSRDNAKDTYYLQMNSLEPEDTADYYCAYGPLTKYGSSWYWPYEYDYWGQGTQVTVSS

SEQ ID NO: 6 - protein, 9 aa, Artificial Sequence
  Re5D06R15 CDR1
ITLDYYAMG

SEQ ID NO: 7 - protein, 15 aa, Artificial Sequence
  Re5D06R15 CDR2
ARIRNSDGSTNYADS

SEQ ID NO: 8 - protein, 19 aa, Artificial Sequence
  Re5D06R15 CDR3
YGPLTKYGSSWYWPYEYDY

SEQ ID NO: 9 - protein, 130 aa, Artificial Sequence
  Re6H06
QVQLVESGGGLVQPGGSLRLSCAASGVTLDYYAIGWFRQAPGKEREGVSCTSSSDGSTYYADSVKGRFTISRDNAKNTVYLQMNSLKPEDTGVYYCAVVPQTYYGGKYYSQCTANGMDYWGKGTLVTVSS

SEQ ID NO: 10 - protein, 9 aa, Artificial Sequence
  Re6H06 CDR1
VTLDYYAIG

SEQ ID NO: 11 - protein, 15 aa, Artificial Sequence
  Re6H06 CDR2
SCTSSSDGSTYYADS

SEQ ID NO: 12 - protein, 22 aa, Artificial Sequence
  Re6H06 CDR3
VVPQTYYGGKYYSQCTANGMDY

SEQ ID NO: 13 - protein, 130 aa, Artificial Sequence
  Re9B09
QVQLVESGGGLVQPGGSLRLSCAASGFTLDYYAIGWFRQAPGKEREGVSRISSSDGSTDYADSVKGRFTISRDNAKNTVYLQMNSLKPEDTAVYYCATVPGTYYSGNWYYTWHPEAVDYWGKGTQVTVSS

SEQ ID NO: 14 - protein, 9 aa, Artificial Sequence
  Re9B09 CDR1
FTLDYYAIG

SEQ ID NO: 15 - protein, 15 aa, Artificial Sequence
  Re9B09 CDR2
SRISSSDGSTDYADS

SEQ ID NO: 16 - protein, 22 aa, Artificial Sequence
  Re9B09 CDR3
TVPGTYYSGNWYYTWHPEAVDY

SEQ ID NO: 17 - protein, 130 aa, Artificial Sequence
  Re31A08
QVQLVESGGGLVQPGGSLRLSCAASGITLDYYSIGWFRQAPGKEREGVSCTSSRDDSTDYADSVKGRFTISRDNAKNSVYLQMNSLNPEDTAVYYCALTPATYYSGRYYFQCPPHGMDYWGKGTLVTVSS

SEQ ID NO: 18 - protein, 9 aa, Artificial Sequence
  Re31A08 CDR1
ITLDYYSIG

SEQ ID NO: 19 - protein, 15 aa, Artificial Sequence
  Re31A08 CDR2
SCTSSRDDSTDYADS

SEQ ID NO: 20 - protein, 22 aa, Artificial Sequence
  Re31A08 CDR3
LTPATYYSGRYYFQCPPHGMDY

SEQ ID NO: 21 - protein, 130 aa, Artificial Sequence
  Re31A12
QVQLVESGGGLVQSGGSLRLSCLTSGVTLDYYAIGWFRQAPGKEREGVSCTSSSDGSTNYSDSVKGRFIISRDNAKNTVYLQMNSLKPEDTAVYYCAVTPATYYGGRYYFQCPYHDMHYWGKGTLVTVSS

SEQ ID NO: 22 - protein, 9 aa, Artificial Sequence
  Re31A12 CDR1
VTLDYYAIG

SEQ ID NO: 23 - protein, 15 aa, Artificial Sequence
  Re31A12 CDR2
SCTSSSDGSTNYSDS

SEQ ID NO: 24 - protein, 22 aa, Artificial Sequence
  Re31A12 CDR3
VTPATYYGGRYYFQCPYHDMHY

SEQ ID NO: 25 - protein, 130 aa, Artificial Sequence
  Ma02H07
QVQLVESGGGLVQPGGSLRLSCAYSGITLDYYAIGWFRQAPGKEREGVSYISSSNDRTDYADSVKGRFTISRDNAKNTVFLQMNSLQPEDTAVYYCATVTGTYYSGRWYYNWHPEAVDYWGKGTLVTVSS

SEQ ID NO: 26 - protein, 9 aa, Artificial Sequence
  Ma02H07 CDR1
ITLDYYAIG

SEQ ID NO: 27 - protein, 15 aa, Artificial Sequence
  Ma02H07 CDR2
SYISSSNDRTDYADS

SEQ ID NO: 28 - protein, 22 aa, Artificial Sequence
  Ma02H07 CDR3
TVTGTYYSGRWYYNWHPEAVDY

SEQ ID NO: 29 - protein, 130 aa, Artificial Sequence
  Ma02F10
QVQLVESGGGLVQPGGSLRLSCAYSGITLDYYAIGWFRQAPGKEREGVSYISGSNDRTDYADSVKGRFTISRDNAKNTVFLQMNSLEPEDTAVYYCATVTGTYYSGRWYYNWHPEAVDYWGKGTLVTVSS

SEQ ID NO: 30 - protein, 9 aa, Artificial Sequence
  Ma02F10 CDR1
ITLDYYAIG

SEQ ID NO: 31 - protein, 15 aa, Artificial Sequence
  Ma02F10 CDR2
SYISGSNDRTDYADS

SEQ ID NO: 32 - protein, 22 aa, Artificial Sequence
  Ma02F10 CDR3
TVTGTYYSGRWYYNWHPEAVDY

SEQ ID NO: 33 - protein, 130 aa, Artificial Sequence
  Ma02E06
QVQLVESGGDLVQPRGSLRLSCAASGITLDYYAIGWFRQAPGKEREGVSYISNTNDKTDYADSVKGRFTISRDNAENTVFLQMNSLQPEDTAVYYCATVPGTYYGGRWYYTWHPEAVRYWGKGTQVTVSS

SEQ ID NO: 34 - protein, 9 aa, Artificial Sequence
  Ma02E06 CDR1
ITLDYYAIG

SEQ ID NO: 35 - protein, 15 aa, Artificial Sequence
  Ma02E06 CDR2
SYISNTNDKTDYADS

SEQ ID NO: 36 - protein, 22 aa, Artificial Sequence
  Ma02E06 CDR3
TVPGTYYGGRWYYTWHPEAVRY

SEQ ID NO: 37 - protein, 128 aa, Artificial Sequence
  Re32D03
QVQLVESGGGLVQPGGSLRLSCAISGITLDYYAVGWFLQAPGKEREGISCMRNWDGRTVYAPSVKGRFTISSDNAKKMVYLEMDNLKSEDTGVYYCAAGPLPPGISCRIPTPLGYDDWGQGTQVTVSS

SEQ ID NO: 38 - protein, 9 aa, Artificial Sequence
  Re32D03 CDR1
ITLDYYAVG

SEQ ID NO: 39 - protein, 15 aa, Artificial Sequence
  Re32D03 CDR2
SCMRNWDGRTVYAPS

SEQ ID NO: 40 - protein, 20 aa, Artificial Sequence
  Re32D03 CDR3
AGPLPPGISCRIPTPLGYDD

SEQ ID NO: 41 - protein, 128 aa, Artificial Sequence
  Re32G06
QVQLVESGGGLVQPGGSLRLSCAISGITLDYYAVGWFLQAPGKEREGISCMRNWDGRTVYAPSVKGRFTISSDNAKKMVYLEMNSLKSEDTGVYYCAAGPLPPGTSCRIPTPLGYDDWGQGTQVTVSS

SEQ ID NO: 42 - protein, 9 aa, Artificial Sequence
  Re32G06 CDR1
ITLDYYAVG

SEQ ID NO: 43 - protein, 15 aa, Artificial Sequence
  Re32G06 CDR2
SCMRNWDGRTVYAPS

SEQ ID NO: 44 - protein, 20 aa, Artificial Sequence
  Re32G06 CDR3
AGPLPPGTSCRIPTPLGYDD

SEQ ID NO: 45 - protein, 128 aa, Artificial Sequence
  Re32B11
QVQLVESGGGLVQPGGSLRLSCATSGITLDYYAIGWFLQAPGKEREGVSCMRNSDGRTVYAPSVKGRFTISRDNAKKMVYLEMNNLKSEDTGVYYCAAGPLPPGISCRIPTPLGYDDWGQGTQVTVSS

SEQ ID NO: 46 - protein, 9 aa, Artificial Sequence
  Re32B11 CDR1
ITLDYYAIG

SEQ ID NO: 47 - protein, 15 aa, Artificial Sequence
  Re32B11 CDR2
SCMRNSDGRTVYAPS

SEQ ID NO: 48 - protein, 20 aa, Artificial Sequence
  Re32B11 CDR3
AGPLPPGISCRIPTPLGYDD

SEQ ID NO: 49 - protein, 128 aa, Artificial Sequence
  Re32A10
QVQLVESGGGLVQPGGSLRLSCATSGITLDYYAIGWFLQAPGKEREGVSCMRSSDGSTVYAPSVKGRFTISRDNAKKMVYLEMNSLKSEDTGVYYCAAGPLPPGTSCRIPTPLGYDDWGQGTQVTVSS

SEQ ID NO: 50 - protein, 9 aa, Artificial Sequence
  Re32A10 CDR1
ITLDYYAIG

SEQ ID NO: 51 - protein, 15 aa, Artificial Sequence
  Re32A10 CDR2
SCMRSSDGSTVYAPS

SEQ ID NO: 52 - protein, 20 aa, Artificial Sequence
  Re32A10 CDR3
AGPLPPGTSCRIPTPLGYDD

SEQ ID NO: 53 - protein, 128 aa, Artificial Sequence; identical to SEQ ID NO: 49
  Re32B02

SEQ ID NO: 54 - protein, 9 aa, Artificial Sequence
  Re32B02 CDR1
ITLDYYAIG

SEQ ID NO: 55 - protein, 15 aa, Artificial Sequence
  Re32B02 CDR2
SCMRSSDGSTVYAPS

SEQ ID NO: 56 - protein, 20 aa, Artificial Sequence
  Re32B02 CDR3
AGPLPPGTSCRIPTPLGYDD

SEQ ID NO: 57 - protein, 128 aa, Artificial Sequence
  Re32F03
QVQLVESGGGLVQPGGSLRLSCATSGITLDYYAIGWFLQAPGKEREGVACMRSSDERSLYAPSVKGRFTISRDNAKKTVYLEMNSLKPEDTGVYYCASGSVVPGTMCRIPTPLGYDDWGQGTQVTVSS

SEQ ID NO: 58 - protein, 9 aa, Artificial Sequence
  Re32F03 CDR1
ITLDYYAIG

SEQ ID NO: 59 - protein, 15 aa, Artificial Sequence
  Re32F03 CDR2
ACMRSSDERSLYAPS

SEQ ID NO: 60 - protein, 20 aa, Artificial Sequence
  Re32F03 CDR3
SGSVVPGTMCRIPTPLGYDD

SEQ ID NO: 61 - protein, 128 aa, Artificial Sequence
  Re32C08
QVQLVESGGGLVQPGGSLRLSCETSGITLDYYAIGWFLQAPGKEREGVACMRNWDGSTVYAPSVKGRFTISRDNDKKAAYLEMNSLKSEDTGVYYCAAGPLPPGHSCRIPTPLGYDDWGQGTQVTVSS

SEQ ID NO: 62 - protein, 9 aa, Artificial Sequence
  Re32C08 CDR1
ITLDYYAIG

SEQ ID NO: 63 - protein, 15 aa, Artificial Sequence
  Re32C08 CDR2
ACMRNWDGSTVYAPS

SEQ ID NO: 64 - protein, 20 aa, Artificial Sequence
  Re32C08 CDR3
AGPLPPGHSCRIPTPLGYDD

SEQ ID NO: 65 - protein, 128 aa, Artificial Sequence
  Re32G01
QVQLVESGGGLVQPGGSLRLSCETSGITLDYYAIGWFLQAPGKDREGVACMRNWDGSTLYAPSVKGRFTISRDADKEVAYLEMNSLKSEDTGVYYCAAGPLPPGHSCRIPTPLGYDDWGQGTQVTVSS

SEQ ID NO: 66 - protein, 9 aa, Artificial Sequence
  Re32G01 CDR1
ITLDYYAIG

SEQ ID NO: 67 - protein, 15 aa, Artificial Sequence
  Re32G01 CDR2
ACMRNWDGSTLYAPS

SEQ ID NO: 68 - protein, 20 aa, Artificial Sequence
  Re32G01 CDR3
AGPLPPGHSCRIPTPLGYDD

SEQ ID NO: 69 - protein, 128 aa, Artificial Sequence
  Re32F02
QVQLVESGGGLVSPGGSLKLSCAASGLTLDYYGIGWFRQVPGKEREGVSCLGVPDNRTLYAPSVKGRFTISRDNAKNTYYLEMNSLNPEDSAVYYCAAGPVVPGHMCRIPTPLGYDYWGQGTLVTVSS

SEQ ID NO: 70 - protein, 9 aa, Artificial Sequence
  Re32F02 CDR1
LTLDYYGIG

SEQ ID NO: 71 - protein, 15 aa, Artificial Sequence
  Re32F02 CDR2
SCLGVPDNRTLYAPS

SEQ ID NO: 72 - protein, 20 aa, Artificial Sequence
  Re32F02 CDR3
AGPVVPGHMCRIPTPLGYDY

SEQ ID NO: 73 - protein, 128 aa, Artificial Sequence
  Re32D08
QVQLVESGGGLVSPGGSLKLSCAASGLTLDYYGIGWFRQVPGKEREGVSCLGVPDNRTLYAPSVKGRFTISRDNAKNTFYLEMNSLNPEDSAVYYCAAGPVVPGHMCRIPTPLGYDYWGQGTQVTVSS

SEQ ID NO: 74 - protein, 9 aa, Artificial Sequence
  Re32D08 CDR1
LTLDYYGIG

SEQ ID NO: 75 - protein, 15 aa, Artificial Sequence
  Re32D08 CDR2
SCLGVPDNRTLYAPS

SEQ ID NO: 76 - protein, 20 aa, Artificial Sequence
  Re32D08 CDR3
AGPVVPGHMCRIPTPLGYDY

SEQ ID NO: 77 - protein, 130 aa, Artificial Sequence
  Re30H02
QVQLVESGGDSVQPGDSLRLSCAISGFTLDYYTIGWFRQAPGKEREGVSCIGSSDSSTSYADAVKGRFTISSDNAKNTVYLQMNNLKPEDTAVYYCAAGPATYYGGNWHHTCHANAMHYWGKGTLVTVSS

SEQ ID NO: 78 - protein, 9 aa, Artificial Sequence
  Re30H02 CDR1
FTLDYYTIG

SEQ ID NO: 79 - protein, 15 aa, Artificial Sequence
  Re30H02 CDR2
SCIGSSDSSTSYADA

SEQ ID NO: 80 - protein, 22 aa, Artificial Sequence
  Re30H02 CDR3
AGPATYYGGNWHHTCHANAMHY

SEQ ID NO: 81 - protein, 130 aa, Artificial Sequence
  Re30B09
QVQLVESGGGLVQPGGSLRLSCEISGFTLDYYTIGWFRQAPGKEREGVSCIGSSDSSTSYADAVKGRFTISSDNAKNTVYLQMNNLKPEDTAVYYCAAGPATYYGGNWHHTCHANAMDYWGKGTLVTVSS

SEQ ID NO: 82 - protein, 9 aa, Artificial Sequence
  Re30B09 CDR1
FTLDYYTIG

SEQ ID NO: 83 - protein, 15 aa, Artificial Sequence
  Re30B09 CDR2
SCIGSSDSSTSYADA

SEQ ID NO: 84 - protein, 22 aa, Artificial Sequence
  Re30B09 CDR3
AGPATYYGGNWHHTCHANAMDY

SEQ ID NO: 85 - protein, 130 aa, Artificial Sequence
  Re30A12
QVQLVESGGGLVQPGGSLRLSCAASGVTLDYYTIGWFRQAPGKEREGVSCIGSGDGSTSYADAVKGRFTISNDNAKNTVYLQMNNLKPEDTAVYYCAVGPATYYGGNWHYTCHADAMRDWGKGTLVTVSS

SEQ ID NO: 86 - protein, 9 aa, Artificial Sequence
  Re30A12 CDR1
VTLDYYTIG

SEQ ID NO: 87 - protein, 15 aa, Artificial Sequence
  Re30A12 CDR2
SCIGSGDGSTSYADA

SEQ ID NO: 88 - protein, 22 aa, Artificial Sequence
  Re30A12 CDR3
VGPATYYGGNWHYTCHADAMRD

SEQ ID NO: 89 - protein, 123 aa, Artificial Sequence
  Re30D01
QVQLVESGGGLVQAGGSLRLSCAASGPIFSFNAVDWYRQAPGKQRELVAQIGHHGATNYVDSVKGRFTISKDSAKNTAYLQMDNLKPEDTAVYRCNAFVSINIPQGREEFGYWGQGTQVTVSS

SEQ ID NO: 90 - protein, 9 aa, Artificial Sequence
  Re30D01 CDR1
PIFSFNAVD

SEQ ID NO: 91 - protein, 14 aa, Artificial Sequence
  Re30D01 CDR2
AQIGHHGATNYVDS

SEQ ID NO: 92 - protein, 16 aa, Artificial Sequence
  Re30D01 CDR3
AFVSINIPQGREEFGY

SEQ ID NO: 93 - protein, 132 aa, Artificial Sequence
  Re30A03
QVQLVESGGGLVQPGDSLTLSCATTEVTLDYYGLCWFRQAPGKGREGVACISSVDGATVYADSVKGRFTISRDNSKNTVSLQMNDLSLEDTAVYSCGAGPMTPYGGRWYFSGLLAGNGMHYWGKGTLVTVSS

SEQ ID NO: 94 - protein, 9 aa, Artificial Sequence
  Re30A03 CDR1
VTLDYYGLC

SEQ ID NO: 95 - protein, 15 aa, Artificial Sequence
  Re30A03 CDR2
ACISSVDGATVYADS

SEQ ID NO: 96 - protein, 24 aa, Artificial Sequence
  Re30A03 CDR3
AGPMTPYGGRWYFSGLLAGNGMHY

SEQ ID NO: 97 - protein, 130 aa, Artificial Sequence
  Re30E02
QVQLVESGGGLVQPGGSLRLSCAASGLTLDYYTIGWFRQAPGKEREGVTCIASSDGNTVYADSVKGRFTISRDNAKNTVYLQMNSLKPEDTAVYYCAGGPQTYYGGTYHSTCHENAMDYWGKGTLVTVSS

SEQ ID NO: 98 - protein, 9 aa, Artificial Sequence
  Re30E02 CDR1
LTLDYYTIG

SEQ ID NO: 99 - protein, 15 aa, Artificial Sequence
  Re30E02 CDR2
TCIASSDGNTVYADS

SEQ ID NO: 100 - protein, 22 aa, Artificial Sequence
  Re30E02 CDR3
GGPQTYYGGTYHSTCHENAMDY

SEQ ID NO: 101 - protein, 130 aa, Artificial Sequence
  Re30B06
QVQLVESGGGLVQPGGSLKLSCEHSGFTLDYYTIGWFRQAPGKEREGVGCVGSSDGTTYYSDSVKGRFSISRDDAKNTVYLQMNNLKPEDTAVYYCAGGPQTYYGGRYYTTCHEDAMYHWGKGTLVTVSS

SEQ ID NO: 102 - protein, 9 aa, Artificial Sequence
  Re30B06 CDR1
FTLDYYTIG

SEQ ID NO: 103 - protein, 15 aa, Artificial Sequence
  Re30B06 CDR2
GCVGSSDGTTYYSDS

SEQ ID NO: 104 - protein, 22 aa, Artificial Sequence
  Re30B06 CDR3
GGPQTYYGGRYYTTCHEDAMYH

SEQ ID NO: 105 - protein, 128 aa, Artificial Sequence
  Re32E06
QVQLVESGGGLVQPGGSLRLSCETSGITLDYYAIGWFLQAPGKEREGVACMRNWDGSTLYAPSVKGRFTISRDNDKKAVYLEMNSLKSEDTGVYYCAAGPLPPGHSCRIPTPLGYDDWGQGTQVTVSS

SEQ ID NO: 106 - protein, 9 aa, Artificial Sequence
  Re32E06 CDR1
ITLDYYAIG

SEQ ID NO: 107 - protein, 15 aa, Artificial Sequence
  Re32E06 CDR2
ACMRNWDGSTLYAPS

SEQ ID NO: 108 - protein, 20 aa, Artificial Sequence
  Re32E06 CDR3
AGPLPPGHSCRIPTPLGYDD

SEQ ID NO: 109 - protein, 128 aa, Artificial Sequence
  Ma6F06
QVQLVESGGGLVQPGGSLRLSCATSGITLDYYAIGWFLQVPGKEREGVACMRNWDGSTLYAPSVKGRFTISRDADKEVAYLEMNSLKSEDTGVYYCAAGPLPPGHSCRIPTPLGYDDWGQGTQVTVSS

SEQ ID NO: 110 - protein, 9 aa, Artificial Sequence
  Ma6F06 CDR1
ITLDYYAIG

SEQ ID NO: 111 - protein, 15 aa, Artificial Sequence
  Ma6F06 CDR2
ACMRNWDGSTLYAPS

SEQ ID NO: 112 - protein, 20 aa, Artificial Sequence
  Ma6F06 CDR3
AGPLPPGHSCRIPTPLGYDD

SEQ ID NO: 113 - protein, 231 aa, Artificial Sequence
  wt_RBD-AviHis
ETNLCPFGEVFNATRFASVYAWNRKRISNCVADYSVLYNSASFSTFKCYGVSPTKLNDLCFTNVYADSFVIRGDEVRQIAPGQTGKIADYNYKLPDDFTGCVIAWNSNNLDSKVGGNYNYLYRLFRKSNLKPFERDISTEIYQAGSTPCNGVEGFNCYFPLQSYGFQPTNGVGYQPYRVVVLSFELLHAPATVCGPKTGTGGSGGSGLNDIFEAQKIEWHEGRTKHHHHHH

SEQ ID NO: 114 - protein, 231 aa, Artificial Sequence
  TetraMutRBD-AviHis
ETNLCPFGEVFNATRFASVYAWNRKRISNCVADYSVLYNSASFSTFKCYGVSPTKLNDLCFTNVYADSFVIRGDEVRQIAPGQTGTIADYNYKLPDDFTGCVIAWNSNNLDSKVGGNYNYRYRLFRKSNLKPFERDISTEIYQAGSTPCNGVKGFNCYFPLQSYGFQPTYGVGYQPYRVVVLSFELLHAPATVCGPKTGTGGSGGSGLNDIFEAQKIEWHEGRTKHHHHHH

SEQ ID NO: 115 - protein, 127 aa, Artificial Sequence
  Re9F06
GSQVQLVESGGGLVQAGGSLRLSCAASGRTFSNDALGWFRQAPRKEREFVAAINWNSGTYYADSVKGRFTISRDNAKNTVYLQMNSLKPEDTAVYSCAAASDYGLPREDFLYDYWGQGTQVTVSSTS

SEQ ID NO: 116 - protein, 268 aa, Artificial Sequence
  Re9F06-Re5D06R15_Tandem
EGSQVQLVESGGGLVQAGGSLRLSCAASGRTFSNDALGWFRQAPRKEREFVAAINWNSGTYYADSVKGRFTISRDNAKNTVYLQMNSLKPEDTAVYSCAAASDYGLPREDFLYDYWGQGTQVTVSETEGEGEGGGEGGEGSQVQLVESGGGLVEPGGSLRLSCAASGITLDYYAMGWFREAPGKEREGVARIRNSDGSTNYADSVKGRFTMSRDNAKDTYYLQMNSLEPEDTADYYCAYGPLTKYGSSWYWPYEYDYWGEGTEVTVSS

SEQ ID NO: 117 - protein, 268 aa, Artificial Sequence
  Re9F06-Re5D06R28_Tandem
EGSQVQLVESGGGLVQAGGSLRLSCAASGRTFSNDALGWFRQAPRKEREFVAAINWNSGTYYADSVKGRFTISRDNAKNTVYLQMNSLKPEDTAVYSCAAASDYGLPREDFLYDYWGQGTQVTVSETEGEGEGGGEGGEGSQVQLVESGGGLVEPGGSLRLSCAISGSTLDYYAMGWFREAPGKEREGVARWRNNDGSTNYADSVKGRFTMSRDNAKDTYYLQMNSLEPEDTADYYCAYGPLTKYGSSWHWPYEYDYWGEGTEVTVSS